European Patent Application EP 4 215 618 A1, published July 26, 2023. Title: METHOD FOR MULTI-DIMENSIONAL ANALYSIS OF CELL EPIGENOMICS. Applicant: BGI SHENZHEN. The sequence listing filed with the application follows.

SEQUENCE LISTING (23 sequences)

SEQ ID NO: 1 - DNA, 19 bp, Artificial sequence
ctgtctcttatacacatct

SEQ ID NO: 2 - DNA, 56 bp, Artificial sequence
tcgtcggcagcgtcaggcgaaggcgatcgaggacggcagatgtgtataagagacag

SEQ ID NO: 3 - DNA, 56 bp, Artificial sequence
tcgtcggcagcgtctaatcttagcgatcgaggacggcagatgtgtataagagacag

SEQ ID NO: 4 - DNA, 56 bp, Artificial sequence
tcgtcggcagcgtccaggacgtgcgatcgaggacggcagatgtgtataagagacag

SEQ ID NO: 5 - DNA, 56 bp, Artificial sequence
tcgtcggcagcgtcgtactgacgcgatcgaggacggcagatgtgtataagagacag

SEQ ID NO: 6 - DNA, 59 bp, Artificial sequence
gtctcgtgggctcggaatctatcaacaccgtctccgcctcagatgtgtataagagacag

SEQ ID NO: 7 - DNA, 59 bp, Artificial sequence
gtctcgtgggctcggaccaggaaggcaccgtctccgcctcagatgtgtataagagacag

SEQ ID NO: 8 - DNA, 59 bp, Artificial sequence
gtctcgtgggctcgggagagatattcaccgtctccgcctcagatgtgtataagagacag

SEQ ID NO: 9 - DNA, 59 bp, Artificial sequence
gtctcgtgggctcgggggaaacatgcaccgtctccgcctcagatgtgtataagagacag

SEQ ID NO: 10 - DNA, 56 bp, Artificial sequence
tcgtcggcagcgtctatagcctgcgatcgaggacggcagatgtgtataagagacag

SEQ ID NO: 11 - DNA, 56 bp, Artificial sequence
tcgtcggcagcgtcatagaggcgcgatcgaggacggcagatgtgtataagagacag

SEQ ID NO: 12 - DNA, 56 bp, Artificial sequence
tcgtcggcagcgtccctatcctgcgatcgaggacggcagatgtgtataagagacag

SEQ ID NO: 13 - DNA, 56 bp, Artificial sequence
tcgtcggcagcgtcggctctgagcgatcgaggacggcagatgtgtataagagacag

SEQ ID NO: 14 - DNA, 59 bp, Artificial sequence
gtctcgtgggctcggatttatgacacaccgtctccgcctcagatgtgtataagagacag

SEQ ID NO: 15 - DNA, 59 bp, Artificial sequence
gtctcgtgggctcggccttaattaacaccgtctccgcctcagatgtgtataagagacag

SEQ ID NO: 16 - DNA, 59 bp, Artificial sequence
gtctcgtgggctcggtcagtgagtccaccgtctccgcctcagatgtgtataagagacag

SEQ ID NO: 17 - DNA, 59 bp, Artificial sequence
gtctcgtgggctcggactgccttatcaccgtctccgcctcagatgtgtataagagacag

SEQ ID NO: 18 - DNA, 18 bp, Artificial sequence
cgtagccatgtcgttctg

SEQ ID NO: 19 - DNA, 37 bp, Artificial sequence
gagacgttctcgactcagcagagtctcgtgggctcgg

SEQ ID NO: 20 - DNA, 22 bp, Artificial sequence
gagacgttctcgactcagcaga

SEQ ID NO: 21 - DNA, 24 bp, Artificial sequence
cgagaacgtctccgtagccatgtc

SEQ ID NO: 22 - DNA, 34 bp, Artificial sequence
cgtagccatgtcgttctgcgtcgtcggcagcgtc

SEQ ID NO: 23 - DNA, 37 bp, Artificial sequence; identical to SEQ ID NO: 19